European Patent Specification EP 3 870 594 B1, published August 2, 2023. Title: Process for the purification of oligonucleotides. Applicant: F.Hoffmann- La Roche AG. The sequence listing filed with the application follows.

SEQUENCE LISTING (1 sequence)

SEQ ID NO: 1 - DNA, 17 bp, oligonucleotide sequence
cttctctatctacgcat